European Patent Application EP 4 692 778 A1, published February 11, 2026. Title: ピロリン酸の検出方法. Applicant: デンカ株式会社. Application JP. The sequence listing filed with the application follows.

SEQUENCE LISTING (3 sequences)

SEQ ID NO: 1 - DNA, 48 bp, synthetic construct
  source 1..48: mol_type = other DNA
gcgcgggactggccgtcgttttacaagccgccgccgccgaaccgacac

SEQ ID NO: 2 - DNA, 44 bp, synthetic construct
  source 1..44: mol_type = other DNA
gggactggccgtcgttttacaagccgccgccgccgaaccgacac

SEQ ID NO: 3 - DNA, 21 bp, synthetic construct
  source 1..21: mol_type = other DNA
ttgtaaaacgacggccagtcc